European Patent Application EP 4 364 753 A1, published May 8, 2024. Title: VETERINARY VACCINE COMPOSITION AGAINST HELMINTHS, METHOD FOR TREATMENT AND PREVENTION OF INFECTION CAUSED BY HELMINTHS AND USE. Applicant: FABP Biotech Desenvolvimento em Biotecnologia Ltda. Fundação OSwaldo Cruz. The sequence listing filed with the application follows.

SEQUENCE LISTING (7 sequences)

SEQ ID NO: 1 - protein, 133 aa, Schistosoma mansoni
MSSFLGKWKLSESHNFDAVMSKLGVSWATRQIGNTVTPTVTFTMDGDKMTMLTESTFKNLSCTFKFGEEFDEKTSDGRNVKSVVEKNSESKLTQTQVDPKNTTVIVREVDGDTMKTTVTVGDVTAIRNYKRLS

SEQ ID NO: 2 - protein, 133 aa, Schistosoma mansoni
MSSFLGKWKLSESHNFDAVTSKLGVSWATRQIGNTVTPTVTFTMDGDKMTMLTESTFKNLSCTFKFGEEFDEKTSDGRNVKSVVEKNSESKLTQTQVDPKNTTVIVREVDGDTMKTTVTVGDVTAIRNYKRLS

SEQ ID NO: 3 - protein, 133 aa, Schistosoma mansoni
MSSFLGKWKLSESHNFDAVASKLGVSWATRQIGNTVTPTVTFTMDGDKMTMLTESTFKNLSCTFKFGEEFDEKTSDGRNVKSVVEKNSESKLTQTQVDPKNTTVIVREVDGDTMKTTVTVGDVTAIRNYKRLS

SEQ ID NO: 4 - protein, 133 aa, Schistosoma mansoni
MSSFLGKWKLSESHNFDAVMSKLGVSWATRQIGNTVTPTVTFTMDGDKMTMLTESTFKNLSSTFKFGEEFDEKTSDGRNVKSVVEKNSESKLTQTQVDPKNTTVIVREVDGDTMKTTVTVGDVTAIRNYKRLS

SEQ ID NO: 5 - protein, 133 aa, Schistosoma mansoni
MSSFLGKWKLSESHNFDAVMSKLGVSWATRQIGNTVTPTVTFTMDGDKMTMLTESTFKNLSVTFKFGEEFDEKTSDGRNVKSVVEKNSESKLTQTQVDPKNTTVIVREVDGDTMKTTVTVGDVTAIRNYKRLS

SEQ ID NO: 6 - protein, 132 aa, Fasciola hepatica
MANFVGSWKLEQSENMDAVLQKLGINVIKRKLITSSKPEITFTLEGNKMTMKTVSALKTTVISFTFGEEFKEETADGRTVMTTFTKDSDSKISQVQKCPENTTHVVREVTGGKMIATVTVGDVKAVNNYHKV

SEQ ID NO: 7 - protein, 134 aa, Fasciola hepatica
MSGFIGKWKLVDSRDFDKVMVELGVGYMTRKIAENTKPTVTITKFGEDGLTMKTESTFKTSEISFQFGVEFDETTADGRQVKSTVTKDSDYRITQVQKHPNADTHIVRQVENDIMDTTVTVRDVVSHRRYQRIK